European Patent Specification EP 3 463 444 B1, published October 16, 2024. Title: Improvement of L2 Peptide Immunogenicity. Applicant: Deutsches Krebsforschungszentrum. The sequence listing filed with the application follows.

SEQUENCE LISTING (82 sequences)

SEQ ID NO: 1 - protein, 30 aa, Human papillomavirus
TCKQAGTCPPDIIPKVEGKTIADQILQYGS

SEQ ID NO: 2 - protein, 30 aa, Human papillomavirus
TCKQSGTCPPDVVPKVEGTTLADKILQWSS

SEQ ID NO: 3 - protein, 30 aa, Human papillomavirus
TCKQSGTCPPDVINKVEGTTLADKILQWSS

SEQ ID NO: 4 - protein, 30 aa, Human papillomavirus
TCKAAGTCPSDVIPKIEHTTIADQILRYGS

SEQ ID NO: 5 - protein, 30 aa, Human papillomavirus
TCKATGTCPPDVIPKVEGSTIADQILKYGS

SEQ ID NO: 6 - protein, 30 aa, Human papillomavirus
TCKAAGTCPPDVIPKVEGNTVADQILKYGS

SEQ ID NO: 7 - protein, 30 aa, Human papillomavirus
TCKQAGTCPSDVINKVEGTTLAGKILQWTS

SEQ ID NO: 8 - protein, 30 aa, Human papillomavirus
TCKLSGTCPEDVVNKIEQKTWADKILQWGS

SEQ ID NO: 9 - protein, 30 aa, Human papillomavirus
TCKAAGTCPPDVVNKVEGTTLADKILQWSG

SEQ ID NO: 10 - protein, 30 aa, Human papillomavirus
TCKQSGTCPPDVVDKVEGTTLADKILQWTS

SEQ ID NO: 11 - protein, 30 aa, Human papillomavirus
TCKAAGTCPPDVIPKVKGTTLADKILQWSG

SEQ ID NO: 12 - protein, 30 aa, Human papillomavirus
TCKLTGTCPPDVIPKVEHNTIADQILKWGS

SEQ ID NO: 13 - protein, 19 aa, Human papillomavirus
KTCKQAGTCPPDIIPKVEG

SEQ ID NO: 14 - protein, 19 aa, Human papillomavirus
KTCKQSGTCPPDVVPKVEG

SEQ ID NO: 15 - protein, 19 aa, Human papillomavirus
RTCKQSGTCPPDVINKVEG

SEQ ID NO: 16 - protein, 19 aa, Human papillomavirus
QTCKAAGTCPSDVIPKIEH

SEQ ID NO: 17 - protein, 19 aa, Human papillomavirus
QTCKATGTCPPDVIPKVEG

SEQ ID NO: 18 - protein, 19 aa, Human papillomavirus
RTCKAAGTCPPDVIPKVEG

SEQ ID NO: 19 - protein, 19 aa, Human papillomavirus
KTCKQAGTCPSDVINKVEG

SEQ ID NO: 20 - protein, 19 aa, Human papillomavirus
KTCKLSGTCPEDVVNKIEQ

SEQ ID NO: 21 - protein, 19 aa, Human papillomavirus
STCKAAGTCPPDVVNKVEG

SEQ ID NO: 22 - protein, 19 aa, Human papillomavirus
RTCKQSGTCPPDVVDKVEG

SEQ ID NO: 23 - protein, 19 aa, Human papillomavirus
STCKAAGTCPPDVIPKVKG

SEQ ID NO: 24 - protein, 19 aa, Human papillomavirus
QTCKLTGTCPPDVIPKVEH

SEQ ID NO: 25 - protein, 240 aa, Artificial
  11 mer of peptides from various HPV
KTCKQAGTCPPDIIPKVEGGGPKTCKQSGTCPPDVVPKVEGGGPQTCKAAGTCPSDVIPKIEHGGPQTCKATGTCPPDVIPKVEGGGPRTCKAAGTCPPDVIPKVEGGGPRTCKQSGTCPPDVVDKVEGGGPRTCKQSGTCPPDVINKVEGGGPSTCKAAGTCPPDVVNKVEGGGPKTCKLSGTCPEDVVNKIEQGGPKTCKQAGTCPSDVINKVEGGGPSTCKAAGTCPPDVIPKVKGG

SEQ ID NO: 26 - protein, 174 aa, Artificial
  8mer of peptides from various HPV
KTCKQAGTCPPDIIPKVEGGGPKTCKQSGTCPPDVVPKVEGGGPQTCKAAGTCPSDVIPKIEHGGPQTCKATGTCPPDVIPKVEGGGPRTCKAAGTCPPDVIPKVEGGGPQTCKLTGTCPPDVIPKVEHGGPSTCKAAGTCPPDVVNKVEGGGPKTCKQAGTCPSDVINKVEGG

SEQ ID NO: 27 - protein, 342 aa, Artificial
  PfTrx 11mer
MIIEYDGEIDFTKGRVVLWFSIPGCGPKTCKQAGTCPPDIIPKVEGGGPKTCKQSGTCPPDVVPKVEGGGPQTCKAAGTCPSDVIPKIEHGGPQTCKATGTCPPDVIPKVEGGGPRTCKAAGTCPPDVIPKVEGGGPRTCKQSGTCPPDVVDKVEGGGPRTCKQSGTCPPDVINKVEGGGPSTCKAAGTCPPDVVNKVEGGGPKTCKLSGTCPEDVVNKIEQGGPKTCKQAGTCPSDVINKVEGGGPSTCKAAGTCPPDVIPKVKGGGPCRLVERFMTELSEYFEDIQIVHINAGKWKNIVDKFNILNVPTLVYLKDGREVGRQNLIRSKEEILKKLKELQE

SEQ ID NO: 28 - DNA, 1029 bp, Artificial
  PfTrx 11mer coding
atgattatcgagtatgacggcgaaatcgacttcaccaaaggtcgtgttgtactgtggtttagcattccgggatgcggtccgaagacgtgcaaacaagcgggcacctgtccgcccgatattatcccgaaagtcgagggtggtgggccgaaaacgtgcaaacagtctggaacatgcccgccggatgtggtgccgaaagtggaaggaggaggtccgcaaacgtgcaaagcagcagggacctgtccgtcagatgtgattccgaagattgaacatggtgggccacagacctgtaaagccaccggcacgtgtccgccagacgtaatccctaaagtcgaaggtggtggccctcgtacgtgcaaagctgcgggcacatgccctccggatgttattccgaaagtagaaggcggcggcccacgcacttgcaaacagagtggtacctgcccgccggacgtcgtggataaagttgaaggcggtggtcctcgcacgtgcaagcaaagcggcacatgcccacccgacgtaatcaataaggtcgaaggcggtgggccatcgacttgtaaggcggccgggacttgtccgccagatgtggttaacaaagtggaaggcggcggacctaaaacttgcaaactgagtggaacctgtccggaggatgtagtcaacaaaatcgaacagggcggcccgaaaacctgtaaacaagcaggcacctgtccatcggatgtgattaacaaagttgaaggtggtggtccgagcacgtgtaaagccgctggtacatgccctcccgatgttatccccaaagttaaaggcggcggtccgtgtcgtctggttgaacgcttcatgaccgaactgagcgagtattttgaggatatccaaattgtccatatcaatgccggcaaatggaaaaacatcgtagacaaattcaatattctgaacgtgccgaccctggtatatctgaaagatggccgtgaggttggacgccaaaacctgattcgttctaaagaagagattctgaaaaaactgaaagagctgcaggagtaa

SEQ ID NO: 29 - protein, 276 aa, Artificial
  PfTrx 8mer
MIIEYDGEIDFTKGRVVLWFSIPGCGPKTCKQAGTCPPDIIPKVEGGGPKTCKQSGTCPPDVVPKVEGGGPQTCKAAGTCPSDVIPKIEHGGPQTCKATGTCPPDVIPKVEGGGPRTCKAAGTCPPDVIPKVEGGGPQTCKLTGTCPPDVIPKVEHGGPSTCKAAGTCPPDVVNKVEGGGPKTCKQAGTCPSDVINKVEGGGPCRLVERFMTELSEYFEDIQIVHINAGKWKNIVDKFNILNVPTLVYLKDGREVGRQNLIRSKEEILKKLKELQE

SEQ ID NO: 30 - DNA, 831 bp, Artificial
  PfTrx 8mer coding
atgattatcgagtatgacggcgaaatcgacttcaccaaaggtcgtgttgtactgtggtttagcattccgggatgcggtccgaagacctgtaaacaggccgggacttgcccaccggatattattccaaaggtagaaggtggtggacccaaaacgtgcaaacaaagcgggacgtgcccaccagacgtggtgcccaaagttgaaggcggcgggccgcaaacgtgtaaggccgctggtacgtgcccgagtgatgttattccgaaaattgaacatggtggtccacagacctgtaaagcgaccggcacatgcccgccggatgtgattcctaaagtggaaggtggaggccctcgtacatgcaaggcggctggtacatgcccgcctgatgtcatcccgaaagtcgaaggtggcgggccgcagacgtgcaagttgaccggcacctgtccgccggatgttatcccgaaagttgagcatggcggcccgtctacgtgcaaagcagcagggacctgtccgcctgatgtcgtaaacaaagtcgagggtggcggtcccaaaacctgtaaacaagcgggaacttgtccgtcagacgtcatcaacaaagtagaaggcggcggtccgtgtcgtctggttgaacgcttcatgaccgaactgagcgagtattttgaggatatccaaattgtccatatcaatgccggcaaatggaaaaacatcgtagacaaattcaatattctgaacgtgccgaccctggtatatctgaaagatggccgtgaggttggacgccaaaacctgattcgttctaaagaagagattctgaaaaaactgaaagagctgcaggagtaa

SEQ ID NO: 31 - protein, 387 aa, Artificial
  PADRE2x PfTrx 11mer
MRGDGAKFVAAWTLKAAAGPGPGMIIEYDGEIDFTKGRVVLWFSIPGCGPKTCKQAGTCPPDIIPKVEGGGPKTCKQSGTCPPDVVPKVEGGGPQTCKAAGTCPSDVIPKIEHGGPQTCKATGTCPPDVIPKVEGGGPRTCKAAGTCPPDVIPKVEGGGPRTCKQSGTCPPDVVDKVEGGGPRTCKQSGTCPPDVINKVEGGGPSTCKAAGTCPPDVVNKVEGGGPKTCKLSGTCPEDVVNKIEQGGPKTCKQAGTCPSDVINKVEGGGPSTCKAAGTCPPDVIPKVKGGGPCRLVERFMTELSEYFEDIQIVHINAGKWKNIVDKFNILNVPTLVYLKDGREVGRQNLIRSKEEILKKLKELQEGPGPGAKFVAAWTLKAAAGRGD

SEQ ID NO: 32 - DNA, 1164 bp, Artificial
  PADRE2x PfTrx 11mer coding
atgcgcggcgatggcgccaaattcgttgcggcatggaccctgaaagcggcagcaggccctggaccgggtatgattatcgagtatgacggcgaaatcgacttcaccaaaggtcgtgttgtactgtggtttagcattccgggatgcggtccgaagacgtgcaaacaagcgggcacctgtccgcccgatattatcccgaaagtcgagggtggtgggccgaaaacgtgcaaacagtctggaacatgcccgccggatgtggtgccgaaagtggaaggaggaggtccgcaaacgtgcaaagcagcagggacctgtccgtcagatgtgattccgaagattgaacatggtgggccacagacctgtaaagccaccggcacgtgtccgccagacgtaatccctaaagtcgaaggtggtggccctcgtacgtgcaaagctgcgggcacatgccctccggatgttattccgaaagtagaaggcggcggcccacgcacttgcaaacagagtggtacctgcccgccggacgtcgtggataaagttgaaggcggtggtcctcgcacgtgcaagcaaagcggcacatgcccacccgacgtaatcaataaggtcgaaggcggtgggccatcgacttgtaaggcggccgggacttgtccgccagatgtggttaacaaagtggaaggcggcggacctaaaacttgcaaactgagtggaacctgtccggaggatgtagtcaacaaaatcgaacagggcggcccgaaaacctgtaaacaagcaggcacctgtccatcggatgtgattaacaaagttgaaggtggtggtccgagcacgtgtaaagccgctggtacatgccctcccgatgttatccccaaagttaaaggcggcggtccgtgtcgtctggttgaacgcttcatgaccgaactgagcgagtattttgaggatatccaaattgtccatatcaatgccggcaaatggaaaaacatcgtagacaaattcaatattctgaacgtgccgaccctggtatatctgaaagatggccgtgaggttggacgccaaaacctgattcgttctaaagaagagattctgaaaaaactgaaagagctgcaggagggtccgggtccaggggcgaagtttgtggccgcttggacgttaaaagccgctgcggggcgtggggactaa

SEQ ID NO: 33 - protein, 387 aa, Artificial; identical to SEQ ID NO: 31
  (RGD_PADRE)2x_PfTrx 11mer

SEQ ID NO: 34 - protein, 321 aa, Artificial
  PADRE2x PfTrx 8mer
MRGDGAKFVAAWTLKAAAGPGPGMIIEYDGEIDFTKGRVVLWFSIPGCGPKTCKQAGTCPPDIIPKVEGGGPKTCKQSGTCPPDVVPKVEGGGPQTCKAAGTCPSDVIPKIEHGGPQTCKATGTCPPDVIPKVEGGGPRTCKAAGTCPPDVIPKVEGGGPQTCKLTGTCPPDVIPKVEHGGPSTCKAAGTCPPDVVNKVEGGGPKTCKQAGTCPSDVINKVEGGGPCRLVERFMTELSEYFEDIQIVHINAGKWKNIVDKFNILNVPTLVYLKDGREVGRQNLIRSKEEILKKLKELQEGPGPGAKFVAAWTLKAAAGRGD

SEQ ID NO: 35 - DNA, 966 bp, Artificial
  PADRE2x PfTrx 8mer coding
atgcgcggcgatggcgccaaattcgttgcggcatggaccctgaaagcggcagcaggccctggaccgggtatgattatcgagtatgacggcgaaatcgacttcaccaaaggtcgtgttgtactgtggtttagcattccgggatgcggtccgaagacctgtaaacaggccgggacttgcccaccggatattattccaaaggtagaaggtggtggacccaaaacgtgcaaacaaagcgggacgtgcccaccagacgtggtgcccaaagttgaaggcggcgggccgcaaacgtgtaaggccgctggtacgtgcccgagtgatgttattccgaaaattgaacatggtggtccacagacctgtaaagcgaccggcacatgcccgccggatgtgattcctaaagtggaaggtggaggccctcgtacatgcaaggcggctggtacatgcccgcctgatgtcatcccgaaagtcgaaggtggcgggccgcagacgtgcaagttgaccggcacctgtccgccggatgttatcccgaaagttgagcatggcggcccgtctacgtgcaaagcagcagggacctgtccgcctgatgtcgtaaacaaagtcgagggtggcggtcccaaaacctgtaaacaagcgggaacttgtccgtcagacgtcatcaacaaagtagaaggcggcggtccgtgtcgtctggttgaacgcttcatgaccgaactgagcgagtattttgaggatatccaaattgtccatatcaatgccggcaaatggaaaaacatcgtagacaaattcaatattctgaacgtgccgaccctggtatatctgaaagatggccgtgaggttggacgccaaaacctgattcgttctaaagaagagattctgaaaaaactgaaagagctgcaggagggtccgggtccaggggcgaagtttgtggccgcttggacgttaaaagccgctgcggggcgtggggactaa

SEQ ID NO: 36 - protein, 356 aa, Artificial
  RGD-PADRE-PfTrx(8mer)-IMX
MRGDGAKFVAAWTLKAAAGPGPGMIIEYDGEIDFTKGRVVLWFSIPGCGPKTCKQAGTCPPDIIPKVEGGGPKTCKQSGTCPPDVVPKVEGGGPQTCKAAGTCPSDVIPKIEHGGPQTCKATGTCPPDVIPKVEGGGPRTCKAAGTCPPDVIPKVEGGGPQTCKLTGTCPPDVIPKVEHGGPSTCKAAGTCPPDVVNKVEGGGPKTCKQAGTCPSDVINKVEGGGPCRLVERFMTELSEYFEDIQIVHINAGKWKNIVDKFNILNVPTLVYLKDGREVGRQNLIRSKEEILKKLKELQDGSKKQGDADVCGEVAYIQSVVSDCHVPTAELRTLLEIRKLFLEIQKLKVEGRRRRRS

SEQ ID NO: 37 - DNA, 1074 bp, Artificial
  RGD-PADRE-PfTrx(8mer)-IMX coding
atgcgcggcgatggcgccaaattcgttgcggcatggaccctgaaagcggcagcaggccctggaccgggtatgattatcgagtatgacggcgaaatcgacttcaccaaaggtcgtgttgtactgtggtttagcattccgggatgcggtccgaagacctgtaaacaggccgggacttgcccaccggatattattccaaaggtagaaggtggtggacccaaaacgtgcaaacaaagcgggacgtgcccaccagacgtggtgcccaaagttgaaggcggcgggccgcaaacgtgtaaggccgctggtacgtgcccgagtgatgttattccgaaaattgaacatggtggtccacagacctgtaaagcgaccggcacatgcccgccggatgtgattcctaaagtggaaggtggaggccctcgtacatgcaaggcggctggtacatgcccgcctgatgtcatcccgaaagtcgaaggtggcgggccgcagacgtgcaagttgaccggcacctgtccgccggatgttatcccgaaagttgagcatggcggcccgtctacgtgcaaagcagcagggacctgtccgcctgatgtcgtaaacaaagtcgagggtggcggtcccaaaacctgtaaacaagcgggaacttgtccgtcagacgtcatcaacaaagtagaaggcggcggtccgtgtcgtctggttgaacgcttcatgaccgaactgagcgagtattttgaggatatccaaattgtccatatcaatgccggcaaatggaaaaacatcgtagacaaattcaatattctgaacgtgccgaccctggtatatctgaaagatggccgtgaggttggacgccaaaacctgattcgttctaaagaagagattctgaaaaaactgaaagagctgcaggacggatccaagaaacagggcgatgccgatgtatgcggagaagtggcgtatatccagtctgtggtcagtgattgccatgtgccgacagcggaattacgcactcttctggaaattcgcaaactgtttctggaaattcagaaactgaaggtagagggtcgtcgtcgtcgccgttcataataa

SEQ ID NO: 38 - protein, 320 aa, Artificial
  (RGD_PADRE)2x_PfTrx 8mer
RGDGAKFVAAWTLKAAAGPGPGMIIEYDGEIDFTKGRVVLWFSIPGCGPKTCKQAGTCPPDIIPKVEGGGPKTCKQSGTCPPDVVPKVEGGGPQTCKAAGTCPSDVIPKIEHGGPQTCKATGTCPPDVIPKVEGGGPRTCKAAGTCPPDVIPKVEGGGPQTCKLTGTCPPDVIPKVEHGGPSTCKAAGTCPPDVVNKVEGGGPKTCKQAGTCPSDVINKVEGGGPCRLVERFMTELSEYFEDIQIVHINAGKWKNIVDKFNILNVPTLVYLKDGREVGRQNLIRSKEEILKKLKELQEGPGPGAKFVAAWTLKAAAGRGD

SEQ ID NO: 39 - protein, 374 aa, Artificial
  RGD-PADRE-PfTrx(8mer)-PADRE-IMX
MRGDGAKFVAAWTLKAAAGPGPGMIIEYDGEIDFTKGRVVLWFSIPGCGPKTCKQAGTCPPDIIPKVEGGGPKTCKQSGTCPPDVVPKVEGGGPQTCKAAGTCPSDVIPKIEHGGPQTCKATGTCPPDVIPKVEGGGPRTCKAAGTCPPDVIPKVEGGGPQTCKLTGTCPPDVIPKVEHGGPSTCKAAGTCPPDVVNKVEGGGPKTCKQAGTCPSDVINKVEGGGPCRLVERFMTELSEYFEDIQIVHINAGKWKNIVDKFNILNVPTLVYLKDGREVGRQNLIRSKEEILKKLKELQDGSGPGAKFVAAWTLKAAAGSKKQGDADVCGEVAYIQSVVSDCHVPTAELRTLLEIRKLFLEIQKLKVEGRRRRRS

SEQ ID NO: 40 - DNA, 1128 bp, Artificial
  RGD-PADRE-PfTrx(8mer)-PADRE-IMX coding
atgcgcggcgatggcgccaaattcgttgcggcatggaccctgaaagcggcagcaggccctggaccgggtatgattatcgagtatgacggcgaaatcgacttcaccaaaggtcgtgttgtactgtggtttagcattccgggatgcggtccgaagacctgtaaacaggccgggacttgcccaccggatattattccaaaggtagaaggtggtggacccaaaacgtgcaaacaaagcgggacgtgcccaccagacgtggtgcccaaagttgaaggcggcgggccgcaaacgtgtaaggccgctggtacgtgcccgagtgatgttattccgaaaattgaacatggtggtccacagacctgtaaagcgaccggcacatgcccgccggatgtgattcctaaagtggaaggtggaggccctcgtacatgcaaggcggctggtacatgcccgcctgatgtcatcccgaaagtcgaaggtggcgggccgcagacgtgcaagttgaccggcacctgtccgccggatgttatcccgaaagttgagcatggcggcccgtctacgtgcaaagcagcagggacctgtccgcctgatgtcgtaaacaaagtcgagggtggcggtcccaaaacctgtaaacaagcgggaacttgtccgtcagacgtcatcaacaaagtagaaggcggcggtccgtgtcgtctggttgaacgcttcatgaccgaactgagcgagtattttgaggatatccaaattgtccatatcaatgccggcaaatggaaaaacatcgtagacaaattcaatattctgaacgtgccgaccctggtatatctgaaagatggccgtgaggttggacgccaaaacctgattcgttctaaagaagagattctgaaaaaactgaaagagctgcaggacggatccggtccaggggcgaagtttgtggccgcttggacgttaaaagccgctgccggatccaagaaacagggcgatgccgatgtatgcggagaagtggcgtatatccagtctgtggtcagtgattgccatgtgccgacagcggaattacgcactcttctggaaattcgcaaactgtttctggaaattcagaaactgaaggtagagggtcgtcgtcgtcgccgttcataataa

SEQ ID NO: 41 - protein, 399 aa, Artificial
  PfTrx 11mer-IMX313T
MIIEYDGEIDFTKGRVVLWFSIPGCGPKTCKQAGTCPPDIIPKVEGGGPKTCKQSGTCPPDVVPKVEGGGPQTCKAAGTCPSDVIPKIEHGGPQTCKATGTCPPDVIPKVEGGGPRTCKAAGTCPPDVIPKVEGGGPRTCKQSGTCPPDVVDKVEGGGPRTCKQSGTCPPDVINKVEGGGPSTCKAAGTCPPDVVNKVEGGGPKTCKLSGTCPEDVVNKIEQGGPKTCKQAGTCPSDVINKVEGGGPSTCKAAGTCPPDVIPKVKGGGPCRLVERFMTELSEYFEDIQIVHINAGKWKNIVDKFNILNVPTLVYLKDGREVGRQNLIRSKEEILKKLKELQEGSKKQGDADVCGEVAYIQSVVSDCHVPTAELRTLLEIRKLFLEIQKLKVEGRRRRRS

SEQ ID NO: 42 - DNA, 1203 bp, Artificial
  PfTrx 11mer-IMX313T coding
atgattatcgagtatgatggcgagattgacttcaccaaaggtcgcgtcgtactgtggtttagcattcccggttgcggtccgaagacgtgcaaacaagcgggcacctgtccgcccgatattatcccgaaagtcgagggtggtgggccgaaaacgtgcaaacagtctggaacatgcccgccggatgtggtgccgaaagtggaaggaggaggtccgcaaacgtgcaaagcagcagggacctgtccgtcagatgtgattccgaagattgaacatggtgggccacagacctgtaaagccaccggcacgtgtccgccagacgtaatccctaaagtcgaaggtggtggccctcgtacgtgcaaagctgcgggcacatgccctccggatgttattccgaaagtagaaggcggcggcccacgcacttgcaaacagagtggtacctgcccgccggacgtcgtggataaagttgaaggcggtggtcctcgcacgtgcaagcaaagcggcacatgcccacccgacgtaatcaataaggtcgaaggcggtgggccatcgacttgtaaggcggccgggacttgtccgccagatgtggttaacaaagtggaaggcggcggacctaaaacttgcaaactgagtggaacctgtccggaggatgtagtcaacaaaatcgaacagggcggcccgaaaacctgtaaacaagcaggcacctgtccatcggatgtgattaacaaagttgaaggtggtggtccgagcacgtgtaaagccgctggtacatgccctcccgatgttatccccaaagttaaaggcggcggtccgtgccgtcttgtggaacggtttatgaccgagttatccgaatacttcgaggacattcagatcgtgcacattaatgcgggcaaatggaagaacatcgttgacaaattcaacatcctcaatgtccctaccctggtttacctcaaagatggtcgcgaagttgggcgccagaacttgattcgcagcaaagaagagattctgaagaaactgaaagaattgcaagaaggctcgaagaaacagggcgatgccgatgtatgcggagaagtggcgtatatccagtctgtggtcagtgattgccatgtgccgacagcggaattacgcactcttctggaaattcgcaaactgtttctggaaattcagaaactgaaggtagagggtcgtcgtcgtcgccgttcataataa

SEQ ID NO: 43 - protein, 333 aa, Artificial
  PfTrx 8mer-IMX313T
MIIEYDGEIDFTKGRVVLWFSIPGCGPKTCKQAGTCPPDIIPKVEGGGPKTCKQSGTCPPDVVPKVEGGGPQTCKAAGTCPSDVIPKIEHGGPQTCKATGTCPPDVIPKVEGGGPRTCKAAGTCPPDVIPKVEGGGPQTCKLTGTCPPDVIPKVEHGGPSTCKAAGTCPPDVVNKVEGGGPKTCKQAGTCPSDVINKVEGGGPCRLVERFMTELSEYFEDIQIVHINAGKWKNIVDKFNILNVPTLVYLKDGREVGRQNLIRSKEEILKKLKELQEGSKKQGDADVCGEVAYIQSVVSDCHVPTAELRTLLEIRKLFLEIQKLKVEGRRRRRS

SEQ ID NO: 44 - DNA, 1005 bp, Artificial
  PfTrx 8mer-IMX313T coding
atgattatcgagtatgatggcgagattgacttcaccaaaggtcgcgtcgtactgtggtttagcattcccggttgcggtccgaagacctgtaaacaggccgggacttgcccaccggatattattccaaaggtagaaggtggtggacccaaaacgtgcaaacaaagcgggacgtgcccaccagacgtggtgcccaaagttgaaggcggcgggccgcaaacgtgtaaggccgctggtacgtgcccgagtgatgttattccgaaaattgaacatggtggtccacagacctgtaaagcgaccggcacatgcccgccggatgtgattcctaaagtggaaggtggaggccctcgtacatgcaaggcggctggtacatgcccgcctgatgtcatcccgaaagtcgaaggtggcgggccgcagacgtgcaagttgaccggcacctgtccgccggatgttatcccgaaagttgagcatggcggcccgtctacgtgcaaagcagcagggacctgtccgcctgatgtcgtaaacaaagtcgagggtggcggtcccaaaacctgtaaacaagcgggaacttgtccgtcagacgtcatcaacaaagtagaaggcggcggtccgtgccgtcttgtggaacggtttatgaccgagttatccgaatacttcgaggacattcagatcgtgcacattaatgcgggcaaatggaagaacatcgttgacaaattcaacatcctcaatgtccctaccctggtttacctcaaagatggtcgcgaagttgggcgccagaacttgattcgcagcaaagaagagattctgaagaaactgaaagaattgcaagaaggctcgaagaaacagggcgatgccgatgtatgcggagaagtggcgtatatccagtctgtggtcagtgattgccatgtgccgacagcggaattacgcactcttctggaaattcgcaaactgtttctggaaattcagaaactgaaggtagagggtcgtcgtcgtcgccgttcataataa

SEQ ID NO: 45 - protein, 109 aa, Escherichia coli
MGDKIIHLTDDSFDTDVLKADGAILVDFWAEWCGPCKMIAPILDEIADEYQGKLTVAKLNIDQNPGTAPKYGIRGIPTLLLFKNGEVAATKVGALSKGQLKEFLDANLA

SEQ ID NO: 46 - DNA, 330 bp, Escherichia coli
atgggcgataaaattattcacctgactgacgacagttttgacacggatgtactcaaagcggacggggcgatcctcgtcgatttctgggcagagtggtgcggtccgtgcaaaatgatcgccccgattctggatgaaatcgctgacgaatatcagggcaaactgaccgttgcaaaactgaacatcgatcaaaaccctggcactgcgccgaaatatggcatccgtggtatcccgactctgctgctgttcaaaaacggtgaagtggcggcaaccaaagtgggtgcactgtctaaaggtcagttgaaagagttcctcgacgctaacctggcgtga

SEQ ID NO: 47 - protein, 105 aa, Mus musculus
MVKLIESKEAFQEALAAAGDKLVVVDFSATWCGPCKMIKPFFHSLCDKYSNVVFLEVDVDDCQDVAADCEVKCMPTFQFYKKGQKVGEFSGANKEKLEASITEYA

SEQ ID NO: 48 - DNA, 318 bp, Mus musculus
atggtgaagctgatcgagagcaaggaagcttttcaggaggccctggccgccgcgggagacaagcttgtcgtggtggacttctctgctacgtggtgcggtccgtgcaaaatgatcaagcccttcttccattccctctgtgacaagtattccaatgtggtgttccttgaagtggatgtggatgactgccaggatgttgctgcagactgtgaagtcaaatgcatgccgaccttccagttttataaaaagggtcaaaaggtgggggagttctccggtgctaacaaggaaaagcttgaagcctctattactgaatatgcctaa

SEQ ID NO: 49 - protein, 105 aa, Homo sapiens
MVKQIESKTAFQEALDAAGDKLVVVDFSATWCGPCKMIKPFFHSLSEKYSNVIFLEVDVDDCQDVASECEVKCMPTFQFFKKGQKVGEFSGANKEKLEATINELV

SEQ ID NO: 50 - DNA, 318 bp, Homo sapiens
atggtgaagcagatcgagagcaagactgcttttcaggaagccttggacgctgcaggtgataaacttgtagtagttgacttctcagccacgtggtgtgggccttgcaaaatgatcaagcctttctttcattccctctctgaaaagtattccaacgtgatattccttgaagtagatgtggatgactgtcaggatgttgcttcagagtgtgaagtcaaatgcatgccaacattccagttttttaagaagggacaaaaggtgggtgaattttctggagccaataaggaaaagcttgaagccaccattaatgaattagtctaa

SEQ ID NO: 51 - protein, 138 aa, Methanosaeta thermophila
MDELDEIRRKKLEELKRELAARSQGTPTIEYPDRPVLVTDSSIDAGIRQYPVFVVDCWAEWCGPCRAIAPVIDEMARELKGRVVFGKLNVDQNPLTSRKYGITAIPTLLVFRNGRLVDRLVGAYPKQILMSRVRKYLD

SEQ ID NO: 52 - DNA, 417 bp, Methanosaeta thermophila
atggacgagctggacgaaatccgccgtaaaaaactggaagaactgaaacgtgaactggctgcccgtagtcaaggaacaccgacgatcgagtatcctgaccgccctgtactggttactgattctagcattgatgccgggatccgccaatatcctgtctttgtggtggactgttgggctgaatggtgcggtccgtgtcgtgctattgctccggtgatcgatgaaatggcccgtgagctgaaaggacgtgtggtattcgggaaactgaacgtggaccaaaatccgctgacgagtcgtaaatatggcattaccgccatccctacactgctggttttccgtaacggtcgtctggttgatcgcctggttggtgcttatccgaaacaaattctgatgtctcgtgtccgtaaatatctggactag

SEQ ID NO: 53 - protein, 100 aa, Pyrococcus furiosus
MIIEYDGEIDFTKGRVVLWFSIPGCGPCRLVERFMTELSEYFEDIQIVHINAGKWKNIVDKFNILNVPTLVYLKDGREVGRQNLIRSKEEILKKLKELQE

SEQ ID NO: 54 - DNA, 303 bp, Pyrococcus furiosus
atgattatcgagtatgacggcgaaatcgacttcaccaaaggtcgtgttgtactgtggtttagcattccgggatgcggtccgtgtcgtctggttgaacgcttcatgaccgaactgagcgagtattttgaggatatccaaattgtccatatcaatgccggcaaatggaaaaacatcgtagacaaattcaatattctgaacgtgccgaccctggtatatctgaaagatggccgtgaggttggacgccaaaacctgattcgttctaaagaagagattctgaaaaaactgaaagagctgcaggagtaa

SEQ ID NO: 55 - protein, 259 aa, Pyrococcus furiosus
MRKSKELTGIEAHINDNKKEESNVEYFEKLRSALLDGVNKGRSLLKHLPVTRIEGQSFRVDIIKFEDGVRVVKQEYKPIPLLKKKFYVGIRELNDGTYDVSIATKAGELLVKDEESLVIREILSTEGIKKMKLSSWDNPEEALNDLMNALQEASNASAGPFGLIINPKRYAKLLKIYEKSGKMLVEVLKEIFRGGIIVTLNIDENKVIIFANTPAVLDVVVGQDVTLQELGPEGDDVAFLVSEAIGIRIKNPEAIVVLE

SEQ ID NO: 56 - protein, 174 aa, Pyrococcus furiosus
MLSERMLKALNDQLNRELYSAYLYFAMAAYFEDLGLEGFANWMKAQAEEEIGHALRFYNYIYDRNGRVELDEIPKPPKEWESPLKAFEAAYEHEKFISKSIYELAALAEEEKDYSTRAFLEWFINEQVEEEASVKKILDKLKFAKDSPQILFMLDKELSARAPKLPGLLMQGGE

SEQ ID NO: 57 - protein, 13 aa, Artificial
  Pan HLA-DR reactive epitope (PADRE)
AKFVAAWTLKAAA

SEQ ID NO: 58 - protein, 15 aa, Artificial
  p2p30
QYIKANSKFIGITEL

SEQ ID NO: 59 - protein, 17 aa, Artificial
  p25
KLIPNASLIENCTKAEL

SEQ ID NO: 60 - protein, 55 aa, Artificial
  oligomerization sequence
KKQGDADVCGEVAYIQSVVSDCHVPTAELRTLLEIRKLFLEIQKLKVEGRRRRRS

SEQ ID NO: 61 - DNA, 165 bp, Artificial
  Sequence encoding oligomerization polypeptide IMX313T
aagaaacagggcgatgccgatgtatgcggagaagtggcgtatatccagtctgtggtcagtgattgccatgtgccgacagcggaattacgcactcttctggaaattcgcaaactgtttctggaaattcagaaactgaaggtagagggtcgtcgtcgtcgccgttca

SEQ ID NO: 62 - protein, 189 aa, Artificial
  (RGD_PADRE)1x_PfTrx_HPV16_L2(20-38)3
MRGDGAKFVAAWTLKAAAGPGPGMIIEYDGEIDFTKGRVVLWFSIPGCGPKTCKQAGTCPPDIIPKVEGGGPKTCKQAGTCPPDIIPKVEGGGPKTCKQAGTCPPDIIPKVEGGGPCRLVERFMTELSEYFEDIQIVHINAGKWKNIVDKFNILNVPTLVYLKDGREVGRQNLIRSKEEILKKLKELQE

SEQ ID NO: 63 - protein, 211 aa, Artificial
  (RGD_PADRE)2x_PfTrx_HPV16_L2(20-38)3
MRGDGAKFVAAWTLKAAAGPGPGMIIEYDGEIDFTKGRVVLWFSIPGCGPKTCKQAGTCPPDIIPKVEGGGPKTCKQAGTCPPDIIPKVEGGGPKTCKQAGTCPPDIIPKVEGGGPCRLVERFMTELSEYFEDIQIVHINAGKWKNIVDKFNILNVPTLVYLKDGREVGRQNLIRSKEEILKKLKELQEGPGPGAKFVAAWTLKAAAGRGD

SEQ ID NO: 64 - protein, 215 aa, Artificial
  (RGD_p2p30)1x_PfTrx_HPV16_L2(20-38)3
MRGDGQYIKANSKFIGITELGPGFNNFTVSFWLRVPKVSASHLEGPGPGMIIEYDGEIDFTKGRVVLWFSIPGCGPKTCKQAGTCPPDIIPKVEGGGPKTCKQAGTCPPDIIPKVEGGGPKTCKQAGTCPPDIIPKVEGGGPCRLVERFMTELSEYFEDIQIVHINAGKWKNIVDKFNILNVPTLVYLKDGREVGRQNLIRSKEEILKKLKELQE

SEQ ID NO: 65 - protein, 263 aa, Artificial
  (RGD_p2p30)2x_PfTrx_HPV16_L2(20-38)3
MRGDGQYIKANSKFIGITELGPGFNNFTVSFWLRVPKVSASHLEGPGPGMIIEYDGEIDFTKGRVVLWFSIPGCGPKTCKQAGTCPPDIIPKVEGGGPKTCKQAGTCPPDIIPKVEGGGPKTCKQAGTCPPDIIPKVEGGGPCRLVERFMTELSEYFEDIQIVHINAGKWKNIVDKFNILNVPTLVYLKDGREVGRQNLIRSKEEILKKLKELQEGPGPGQYIKANSKFIGITELGPGFNNFTVSFWLRVPKVSASHLEGRGD

SEQ ID NO: 66 - protein, 193 aa, Artificial
  (RGD_p25)1x_PfTrx_HPV16_L2(20-38)3
MRGDGKLIPNASLIENCTKAELGPGPGMIIEYDGEIDFTKGRVVLWFSIPGCGPKTCKQAGTCPPDIIPKVEGGGPKTCKQAGTCPPDIIPKVEGGGPKTCKQAGTCPPDIIPKVEGGGPCRLVERFMTELSEYFEDIQIVHINAGKWKNIVDKFNILNVPTLVYLKDGREVGRQNLIRSKEEILKKLKELQE

SEQ ID NO: 67 - protein, 218 aa, Artificial
  (RGD_p25)2x_PfTrx_HPV16_L2(20-38)3
RGDGKLIPNASLIENCTKAELGPGPGMIIEYDGEIDFTKGRVVLWFSIPGCGPKTCKQAGTCPPDIIPKVEGGGPKTCKQAGTCPPDIIPKVEGGGPKTCKQAGTCPPDIIPKVEGGGPCRLVERFMTELSEYFEDIQIVHINAGKWKNIVDKFNILNVPTLVYLKDGREVGRQNLIRSKEEILKKLKELQEGPGPGKLIPNASLIENCTKAELGRGD

SEQ ID NO: 68 - protein, 211 aa, Artificial
  (RGD_PADRE)2x_PfTrx_HPV51_L2(20-38)3
MRGDGAKFVAAWTLKAAAGPGPGMIIEYDGEIDFTKGRVVLWFSIPGCGPSTCKAAGTCPPDVVNKVEGGGPSTCKAAGTCPPDVVNKVEGGGPSTCKAAGTCPPDVVNKVEGGGPCRLVERFMTELSEYFEDIQIVHINAGKWKNIVDKFNILNVPTLVYLKDGREVGRQNLIRSKEEILKKLKELQEGPGPGAKFVAAWTLKAAAGRGD

SEQ ID NO: 69 - protein, 211 aa, Artificial
  (RGD_PADRE)2x_PfTrx_HPV31_L2(20-38)3
MRGDGAKFVAAWTLKAAAGPGPGMIIEYDGEIDFTKGRVVLWFSIPGCGPQTCKAAGTCPSDVIPKIEHGGPQTCKAAGTCPSDVIPKIEHGGPQTCKAAGTCPSDVIPKIEHGGPCRLVERFMTELSEYFEDIQIVHINAGKWKNIVDKFNILNVPTLVYLKDGREVGRQNLIRSKEEILKKLKELQEGPGPGAKFVAAWTLKAAAGRGD

SEQ ID NO: 70 - protein, 175 aa, Artificial
  EcTrx HPV16 L2(20-38)3
MGDKIIHLTDDSFDTDVLKADGAILVDFWAEWCGPKTCKQAGTCPPDIIPKVEGGGPKTCKQAGTCPPDIIPKVEGGGPKTCKQAGTCPPDIIPKVEGGGPCKMIAPILDEIADEYQGKLTVAKLNIDQNPGTAPKYGIRGIPTLLLFKNGEVAATKVGALSKGQLKEFLDANLA

SEQ ID NO: 71 - protein, 189 aa, Artificial; identical to SEQ ID NO: 62
  PADRE1x PfTrx HPV16 L2(20-38)3

SEQ ID NO: 72 - protein, 211 aa, Artificial; identical to SEQ ID NO: 63
  PADRE2x PfTrx HPV16 L2(20-38)3

SEQ ID NO: 73 - protein, 215 aa, Artificial; identical to SEQ ID NO: 64
  p2p301x PfTrx HPV16 L2(20-38)3

SEQ ID NO: 74 - protein, 263 aa, Artificial; identical to SEQ ID NO: 65
  p2p302x PfTrx HPV16 L2(20-38)3

SEQ ID NO: 75 - protein, 193 aa, Artificial; identical to SEQ ID NO: 66
  p251x PfTrx HPV16 L2(20-38)3

SEQ ID NO: 76 - protein, 219 aa, Artificial
  p252x PfTrx HPV16 L2(20-38)3
MRGDGKLIPNASLIENCTKAELGPGPGMIIEYDGEIDFTKGRVVLWFSIPGCGPKTCKQAGTCPPDIIPKVEGGGPKTCKQAGTCPPDIIPKVEGGGPKTCKQAGTCPPDIIPKVEGGGPCRLVERFMTELSEYFEDIQIVHINAGKWKNIVDKFNILNVPTLVYLKDGREVGRQNLIRSKEEILKKLKELQEGPGPGKLIPNASLIENCTKAELGRGD

SEQ ID NO: 77 - protein, 211 aa, Artificial; identical to SEQ ID NO: 69
  PADRE2x PfTrx HPV31 L2(20-38)3

SEQ ID NO: 78 - protein, 211 aa, Artificial; identical to SEQ ID NO: 68
  PADRE2x PfTrx HPV51 L2(20-38)3

SEQ ID NO: 79 - protein, 223 aa, Artificial
  PfTrx HPV16 L2(20-38)3-IMX313T
MIIEYDGEIDFTKGRVVLWFSIPGCGPKTCKQAGTCPPDIIPKVEGGGPKTCKQAGTCPPDIIPKVEGGGPKTCKQAGTCPPDIIPKVEGGGPCRLVERFMTELSEYFEDIQIVHINAGKWKNIVDKFNILNVPTLVYLKDGREVGRQNLIRSKEEILKKLKELQEGSKKQGDADVCGEVAYIQSVVSDCHVPTAELRTLLEIRKLFLEIQKLKVEGRRRRRS

SEQ ID NO: 80 - protein, 179 aa, Artificial
  PfTrx HPV16 L2(20-38)1-IMX313T
MIIEYDGEIDFTKGRVVLWFSIPGCGPKTCKQAGTCPPDIIPKVEGGGPCRLVERFMTELSEYFEDIQIVHINAGKWKNIVDKFNILNVPTLVYLKDGREVGRQNLIRSKEEILKKLKELQEGSKKQGDADVCGEVAYIQSVVSDCHVPTAELRTLLEIRKLFLEIQKLKVEGRRRRRS

SEQ ID NO: 81 - protein, 127 aa, Artificial
  HPV16 L2(20-38)3-IMX313T
MGGPKTCKQAGTCPPDIIPKVEGGGPKTCKQAGTCPPDIIPKVEGGGPKTCKQAGTCPPDIIPKVEGGGPGSKKQGDADVCGEVAYIQSVVSDCHVPTAELRTLLEIRKLFLEIQKLKVEGRRRRRS

SEQ ID NO: 82 - DNA, 5196 bp, Artificial
  expression vector for TfTrx8mer-IMX3T3
cgctgttttggcggatgagagaagattttcagcctgatacagattaaatcagaacgcagaagcggtctgataaaacagaatttgcctggcggcagtagcgcggtggtcccacctgaccccatgccgaactcagaagtgaaacgccgtagcgccgatggtagtgtggggtctccccatgcgagagtagggaactgccaggcatcaaataaaacgaaaggctcagtcgaaagactgggcctttcgttttatctgttgtttgtcggtgaacgctctcctgagtaggacaaatccgccgggagcggatttgaacgttgcgaagcaacggcccggagggtggcgggcaggacgcccgccataaactgccaggcatcaaattaagcagaaggccatcctgacggatggcctttttgcgtttctacaaactcttactagttacgtagatcgtaatctaactgtcagaccaagtttactcatatatactttagattgatttaaaacttcatttttaatttaaaaggatctaggtgaagatcctttttgataatctcatgaccaaacgatcgccttaacgtgagttttcgttccactgagcgtcagaccccttaataagatgatcttcttgagatcgttttggtctgcgcgtaatctcttgctctgaaaacgaaaaaaccgccttgcagggcggtttttcgaaggttctctgagctaccaactctttgaaccgaggtaactggcttggaggagcgcagtcaccaaaacttgtcctttcagtttagccttaaccggcgcatgacttcaagactaactcctctaaatcaattaccagtggctgctgccagtggtgcttttgcatgtctttccgggttggactcaagacgatagttaccggataaggcgcagcggtcggactgaacggggggttcgtgcatacagtccagcttggagcgaactgcctacccggaactgagtgtcaggcgtggaatgagacaaacgcggccataacagcggaatgacaccggtaaaccgaaaggcaggaacaggagagcgcacgagggagccgccagggggaaacgcctggtatctttatagtcctgtcgggtttcgccaccactgatttgagcgtcagatttcgtgatgcttgtcaggggggcggagcctatggaaaaacggctttgccgcggccctctcacttccctgttaagtatcttcctggcatcttccaggaaatctccgccccgttcgtaagccatttccgctcgccgcagtcgaacgaccgagcgtagcgagtcagtgagcgaggaagcggaatatatcctgtatcacatattctgctgacgcaccggtgcagccttttttctcctgccacatgaagcacttcactgacaccctcatcagtgccaacatagtaagccagtatacactccgctagcgctgaggtctgcctcgtgaagaaggtgttgctgactcataccaggcctgaatcgcccgggcatcatccagccagaaagtgagggagccacggttgatgagagctttgttgtaggtggaccagttggtgattttgaacttttgctttgccacggaacggtctgcgttgtcgggaagatgccggcgccatagtggcgcgtgatctgatccttcaactcagcaaaagttcgatttattcaacaaagccacgttgtgtctcaaaatctctgatgttacattgcacaagataaaaatatatcatcatgaacaataaaactgtctgcttacataaacagtaatacaaggggtgttatgagccatattcaacgggaaacgtcttgcagcaggccgcgattaaattccaacatggatgctgatttatatgggtataaatgggctcgcgataatgtcgggcaatcaggtgcgacaatctatcgattgtatgggaagcccgatgcgccagagttgtttctgaaacatggcaaaggtagcgttgccaatgatgttacagatgagatggtcagactaaactggctgacggaatttatgcctcttccgaccatcaagcattttatccgtactcctgatgatgcatggttactcaccactgcgatcccagggaaaacagcattccaggtattagaagaatatccggattcaggtgaaaatattgttgatgcgctggcagtgttcctgcgccggttgcattcgattcctgtttgtaattgtccttttaactctgatcgcgtatttcgtctcgctcaggcgcaatcacgaatgaataacggtttggttgatgcgagtgattttgatgacgagcgtaatggctggcctgttgaacaagtctggaaagaaatgcataaacttttgccattctcaccggattcagtcgtcactcatggtgatttctcacttgataaccttatttttgacgaggggaaattaataggttgtattgatgttggacgagtcggaatcgcagaccgataccaggatcttgccatcctatggaactgcctcggtgagttttctccttcattacagaaacggctttttcaaaaatatggtattgataatcctgatatgaataaattgcagtttcatttgatgctcgatgagtttttctaatcagaattggttaattggttgtaacactggcagagcattacgctgacttgacgggacggccatagtggcctttgttgaataaataaagcctggggtgcctaatgagtgagctaactcacattaattgcgttgcgctcactgcccgctttccagtcgggaaacctgtcgtgccagctgcattaatgaatcggccaacgcgcggggagaggcggtttgcgtattgggcgccagggtggtttttcttttcaccagtgagacgggcaacagctgattgcccttcaccgcctggccctgagagagttgcagcaagcggtccacgctggtttgccccagcaggcgaaaatcctgtttgatggtggttaacggcgggatataacatgagctgtcttcggtatcgtcgtatcccactaccgagatatccgcaccaacgcgcagcccggactcggtaatggcgcgcattgcgcccagcgccatctgatcgttggcaaccagcatcgcagtgggaacgatgccctcattcagcatttgcatggtttgttgaaaaccggacatggcactccagtcgccttcccgttccgctatcggctgaatttgattgcgagtgagatatttatgccagccagccagacgcagacgcgccgagacagaacttaatgggcccgctaacagcgcgatttgctggtgacccaatgcgaccagatgctccacgcccagtcgcgtaccgtcttcatgggagaaaataatactgttgatgggtgtctggtcagagacatcaagaaataacgccggaacattagtgcaggcagcttccacagcaatggcatcctggtcatccagcggatagttaatgatcagcccactgacgcgttgcgcgagaagattgtgcaccgccgctttacaggcttcgacgccgcttcgttctaccatcgacaccaccacgctggcacccagttgatcggcgcgagatttaatcgccgcgacaatttgcgacggcgcgtgcagggccagactggaggtggcaacgccaatcagcaacgactgtttgcccgccagttgttgtgccacgcggttgggaatgtaattcagctccgccatcgccgcttccactttttcccgcgttttcgcagaaacgtggctggcctggttcaccacgcgggaaacggtctgataagagacaccggcatactctgcgacatcgtataacgttactggtttcacattcaccaccctgaattgactctcttccgggcgctatcatgccataccgcgaaaggttttgcgccattcgatggtgtcaacgtaaatgcatgccgcttcgccttccggccaccagaatagcctgcgattcaaccccttcttcgatctgttttgctacccgttgtagcggaattcggtacctgtacaagggcctcgtgatacgcctcgagatttttataggttaatgtcatgataataatggtttcttagacgtctgcgccgacatcataacggttctggcaaatattctgaaatgagctgttgacaattaatcatcggctcgtataatgtgtggaattgtgagcggataacaatttcacacaggagatatcatatgattattgagtacgatggcgagattgactttaccaagggccgtgtggtgctgtggtttagcattccgggttgcggtccgaagacctgcaaacaggcgggtacctgcccgccggacatcattccgaaagtggaaggtggcggtccgaagacctgcaaacaaagcggtacctgcccgccggatgttgttccgaaagtggagggcggtggcccgcaaacctgcaaggcggcgggtacctgcccgagcgacgttatcccgaagattgaacatggtggcccgcagacctgcaaggcgaccggcacctgcccgccggacgtgatcccgaaggttgagggtggcggtccgcgtacctgcaaagcggcgggcacctgcccgccggatgtgattccgaaggttgaaggcggtggccctcagacttgcaaactgactggcacttgcccgccggacgttattccgaaggttgagcatggtggcccgagcacctgcaaagctgctggaacttgcccgccggatgtggttaacaaggttgaaggtggcggtccgaaaacctgcaagcaagcgggcacctgcccgagcgatgtgattaacaaagttgaaggcggtggcccgtgccgtctggttgagcgtttcatgaccgagctgagcgaatactttgaggacatccaaattgtgcacatcaacgcgggcaagtggaaaaacatcgttgacaagttcaacattctgaacgtgccgaccctggtttatctgaaagatggtcgtgaggtgggtcgtcagaacctgatccgtagcaaagaggagattctgaagaaactgaaagaactgcaggaaggtagcaagaagcaaggcgacgcggatgtgtgcggtgaagttgcgtacatccaaagcgtggttagcgattgccacgttccgaccgcggaactgcgtaccctgctggagattcgtaagctgttcctggaaatccaaaaactgaaggttgaaggtcgtcgtcgtcgtcgtagctaataaggatc